European Patent Specification EP 3 419 672 B1, published April 26, 2023. Title: Gene Therapy for the Treatment of a Retinal Degeneration Disease. Applicant: EyeServ GmbH, Tübingen, Germany. The sequence listing filed with the application follows.

SEQUENCE LISTING (8 sequences)

SEQ ID NO: 1 - DNA, 848 bp, Artificial Sequence
  hRHO promoter nucleotide sequence
gctagcagatcttccccacctagccacctggcaaactgctccttctctcaaaggcccaaacatggcctcccagactgcaacccccaggcagtcaggccctgtctccacaacctcacagccaccctggacggaatctgcttcttcccacatttgagtcctcctcagcccctgagctcctctgggcagggctgtttctttccatctttgtattcccaggggcctgcaaataaatgtttaatgaacgaacaagagagtgaattccaattccatgcaacaaggattgggctcctgggccctaggctatgtgtctggcaccagaaacggaagctgcaggttgcagcccctgccctcatggagctcctcctgtcagaggagtgtggggactggatgactccagaggtaacttgtgggggaacgaacaggtaaggggctgtgtgacgagatgagagactgggagaataaaccagaaagtctctagctgtccagaggacatagcacagaggcccatggtccctatttcaaacccaggccaccagactgagctgggaccttgggacagacaagtcatgcagaagttaggggaccttctcctcccttttcctggatcctgagtacctctcctccctgacctcaggcttcctcctagtgtcaccttggcccctcttagaagccaattaggccctcagtttctgcagcggggattaatatgattatgaacacccccaatctcccagatgctgattcagccaggagcttaggagggggaggtcactttataagggtctgggggggtcagaacccagagtcatccgcctgaattctgcagatatccatcacactggcggccg

SEQ ID NO: 2 - DNA, 2581 bp, Artificial Sequence
  hPDE6A nucleotide sequence
atgggcgaggtgacagcagaggaggtggagaagttcctggactcgaatattggctttgccaaacagtactacaacctccactaccgggccaagctcatctccgacctccttggggccaaggaggctgccgtggacttcagcaactaccactccccgagcagcatggaggagagcgaaatcatctttgatctcctgcgggactttcaggagaatttacagacagagaaatgcatcttcaatgtcatgaagaagctgtgcttcctcctgcaggcagaccgcatgagcctgttcatgtaccggacccgcaatggcatcgcagagctggccaccaggcttttcaatgtccacaaggatgctgtcctcgaggactgcctggtgatgcccgaccaagagatcgtcttccctttggacatgggcatcgtgggccatgtcgcacactctaagaaaattgctaacgtccccaacacagaggaggatgagcatttctgtgactttgtggacatcctcacagagtacaagaccaagaacatcttggcttcccccataatgaatgggaaggatgtggtggccataatcatggctgtgaataaagtggatggatcccacttcaccaagagagatgaagagattcttctcaagtacctcaattttgcaaatctaatcatgaaggtgtaccacctgagttacctgcacaactgtgaaactcgacgtggccagatactgctgtggtctgggagcaaagtctttgaagaacttacggacatcgaacgacagttccacaaagccctgtacacagtccgtgctttcctcaactgtgacagatactctgtgggtctcttagacatgaccaagcagaaggaattttttgatgtgtggccggttctgatgggtgaagttccaccttactctggtcccaggactccggatggaagagaaattaacttttacaaggtcattgactacatcctgcatggcaaagaggacatcaaagtcatcccgaatccacctcctgaccattgggctttagtaagcggtctcccagcttatgttgcccagaatggcctgatttgcaacatcatgaatgcgcctgcggaggacttttttgcatttcagaaagaacctctggatgagtctggatggatgattaaaaatgtgctttcaatgccgattgtgaacaagaaggaagaaattgttggagtggccacattttacaatcgtaaagatgggaagccctttgatgaaatggatgagacgctcatggagtctttgactcaatttctgggctggtctgtcttaaatcctgacacctatgagtcaatgaataaacttgaaaataggaaggatattttccaggacatagtaaaatatcatgtgaagtgtgacaatgaagaaattcagaaaatcttgaaaaccagagaggtgtatgggaaggagccatgggagtgtgaggaagaggagctggctgagatcctgcaagcggagctgccagatgcagataaatacgaaattaataaatttcacttcagtgacttacccctaacagaactggagctggtaaaatgtggaatacagatgtattatgagctcaaagtggtggataaatttcacattccacaagaggccctggtgcggttcatgtactccctgagtaagggctaccgcaagatcacctaccacaactggcggcacggcttcaacgtggggcagaccatgttctccctgctggtgacgggaaagctgaagcgctacttcacggacctagaggccttggccatggtcactgctgctttctgccatgacattgaccacagaggcaccaataacctctaccagatgaaatcccagaacccactggccaagctccatgggtcctctatcttggaaagacaccacttggagtttggcaaaacactgctcagagacgagagcctgaatatctttcaaaacctcaatcgtcgacagcatgagcatgccatccacatgatggacattgcaatcattgccacagacctcgccctgtatttcaagaagaggacgatgttccaaaagatcgtggatcagtctaagacatatgagagtgaacaggagtggacacagtacatgatgctggagcagacacggaaggaaatcgttatggccatgatgatgaccgcctgtgatctctcagccatcaccaaaccctgggaggtgcagagccaggtagctctgctggtggctgctgaattctgggaacaaggtgacctggagcgcacggtgctgcaacagaatcccattcccatgatggacagaaacaaagcagatgaactccctaagcttcaagtcggcttcattgactttgtttgcaccttcgtctacaaggaattctcccgtttccacgaggagatcaccccaatgttggacgggatcaccaacaatcgcaaggagtggaaggcgcttgctgatgagtacgatgccaagatgaaggtgcaggaggagaagaagcagaaacagcagtcggccaagtcagcagccgcaggaaatcagccggggggaaaccccagcccagggggtgcaactacatccaagtcctgctgcatccagt

SEQ ID NO: 3 - protein, 860 aa, Artificial Sequence
  hPDE6A amino acid sequence
MGEVTAEEVEKFLDSNIGFAKQYYNLHYRAKLISDLLGAKEAAVDFSNYHSPSSMEESEIIFDLLRDFQENLQTEKCIFNVMKKLCFLLQADRMSLFMYRTRNGIAELATRLFNVHKDAVLEDCLVMPDQEIVFPLDMGIVGHVAHSKKIANVPNTEEDEHFCDFVDILTEYKTKNILASPIMNGKDVVAIIMAVNKVDGSHFTKRDEEILLKYLNFANLIMKVYHLSYLHNCETRRGQILLWSGSKVFEELTDIERQFHKALYTVRAFLNCDRYSVGLLDMTKQKEFFDVWPVLMGEVPPYSGPRTPDGREINFYKVIDYILHGKEDIKVIPNPPPDHWALVSGLPAYVAQNGLICNIMNAPAEDFFAFQKEPLDESGWMIKNVLSMPIVNKKEEIVGVATFYNRKDGKPFDEMDETLMESLTQFLGWSVLNPDTYESMNKLENRKDIFQDIVKYHVKCDNEEIQKILKTREVYGKEPWECEEEELAEILQAELPDADKYEINKFHFSDLPLTELELVKCGIQMYYELKVVDKFHIPQEALVRFMYSLSKGYRKITYHNWRHGFNVGQTMFSLLVTGKLKRYFTDLEALAMVTAAFCHDIDHRGTNNLYQMKSQNPLAKLHGSSILERHHLEFGKTLLRDESLNIFQNLNRRQHEHAIHMMDIAIIATDLALYFKKRTMFQKIVDQSKTYESEQEWTQYMMLEQTRKEIVMAMMMTACDLSAITKPWEVQSQVALLVAAEFWEQGDLERTVLQQNPIPMMDRNKADELPKLQVGFIDFVCTFVYKEFSRFHEEITPMLDGITNNRKEWKALADEYDAKMKVQEEKKQKQQSAKSAAAGNQPGGNPSPGGATTSKSCCIQ

SEQ ID NO: 4 - DNA, 543 bp, Artificial Sequence
  WPREm nucleotide sequence
aatcaacctctggattacaaaatttgtgaaagattgactggtattcttaactatgttgctccttttacgctatgtggatacgctgctttaatgcctttgtatcatgctattgcttcccgtatggctttcattttctcctccttgtataaatcctggttgctgtctctttatgaggagttgtggcccgttgtcaggcaacgtggcgtggtgtgcactgtgtttgctgacgcaacccccactggttggggcattgccaccacctgtcagctcctttccgggactttcgctttccccctccctattgccacggcggaactcatcgccgcctgccttgcccgctgctggacaggggctcggctgttgggcactgacaattccgtggtgttgtcggggaagctgacgtcctttccagggctgctcgcctgtgttgccacctggattctgcgcgggacgtccttctgctacgtcccttcggccctcaatccagcggaccttccttcccgcggcctgctgccggctctgcggcctcttccgcgtcttcga

SEQ ID NO: 5 - DNA, 208 bp, Artificial Sequence
  BGH pA nucleotide sequence
ctgtgccttctagttgccagccatctgttgtttgcccctcccccgtgccttccttgaccctggaaggtgccactcccactgtcctttcctaataaaatgaggaaattgcatcgcattgtctgagtaggtgtcattctattctggggggtggggtggggcaggacagcaagggggaggattgggaagacaatagcaggcatgctgggga

SEQ ID NO: 6 - DNA, 130 bp, Artificial Sequence
  L-ITR nucleotide sequence
ctgcgcgctcgctcgctcactgaggccgcccgggcaaagcccgggcgtcgggcgacctttggtcgcccggcctcagtgagcgagcgagcgcgcagagagggagtggccaactccatcactaggggttcct

SEQ ID NO: 7 - DNA, 130 bp, Artificial Sequence
  R-ITR nucleotide sequence
aggaacccctagtgatggagttggccactccctctctgcgcgctcgctcgctcactgaggccgggcgaccaaaggtcgcccgacgcccgggctttgcccgggcggcctcagtgagcgagcgagcgcgcag

SEQ ID NO: 8 - DNA, 5591 bp, Artificial Sequence
  pGL2.KanR vector backbone nucleotide sequence
tgggcctcagtgagcgagcgagcgcgcagctgcattaatgaatcggccaacgcgcggggagaggcggtttgcgtattgggcgctcttccgcttcctcgctcactgactcgctgcgctcggtcgttcggctgcggcgagcggtatcagctcactcaaaggcggtaatacggttatccacagaatcaggggataacgcaggaaagaacatgtcgcgttgctggcgtttttccataggctccgcccccctgacgagcatcacaaaaatcgacgctcaagtcagaggtggcgaaacccgacaggactataaagataccaggcgtttccccctggaagctccctcgtgcgctctcctgttccgaccctgccgcttaccggatacctgtccgcctttctcccttcgggaagcgtggcgctttctcatagctcacgctgtaggtatctcagttcggtgtaggtcgttcgctccaagctgggctgtgtgcacgaaccccccgttcagcccgaccgctgcgccttatccggtaactatcgtcttgagtccaacccggtaagacacgacttatcgccactggcagcagccactggtaacaggattagcagagcgaggtatgtaggcggtgctacagagttcttgaagtggtggcctaactacggctacactagaagaacagtatttggtatctgcgctctgctgaagccagttaccttcggaaaaagagttggtagctcttgatccggcaaacaaaccaccgctggtagcggtggtttttttgtttgcaagcagcagattacgcgcagaaaaaaaggatctcaagaagatcctttgatcttttctacggggtctgacgctcagtggaacgaaaactcacgttaagggattttggtcatgactgtggaatgtgtgtcagttaggcgacataggtgatctatgtagaagcctagtggaacaggttagtttgagtagctttagaatgtaaattctgggatcatagtgtagtaatctctaattaacggtgacggtttgtaagacaggtcttcgcaaaatcaagcggcaggtgatttcaacagattcttgctgatggtttaggcgtacaatgccctgaagaataagtaagagaatagcactcctcgtcgcctagaattacctaccggcgtccaccataccttcgattatcgcgcccactctcccattagtcggcacaggtggatgtgttgcgatagcccgctaagatattctaaggcgtaacgcagatgaatattctacagagttgccataggcgttgaacgcttcacggacgataggaatgttgcgtatagagcgtgagtcatcgaagtggtgtatacactcgtacttaacatctagcccggctctatcagtacaccagtgccttgaatgacatactcatcattaaactttctcaacagtcaaacgaccaagtgcatttccaaggagtgcgaaggagattcattctctcgccagcactgtaataggcactaaaagagtgaagataagctagagtgccgtgctaagacggtgtcggaacaaagcggtcttacggtcagtcgtatttcctgtcgagtcccgtccagttgagcgtatcactcccagtgtactagcaagccgagaaggctgtgcttggagtcaatcggatgtaggatggtctccagacaccgggccaccactcttcacgcctagaagcatagaacgtcgagcagacatcaaagtcttagtaccggacgtgccgtttcactgcgaatattacctgaagctgtaccgttattgcggagcaaagtgacagtgctgctcttatcatatttgtattgacgacagccgccttcgcggtttcctcagactctagatcgaatacaggcttattgtaggcagaggcacgcccttgttagtggctgcggcaatatcttccgatccccttgtctaaccatgaatcaattctctcatttgaagaccctaatatgtcatcattagtgtttcaaatgccaccaaataccgcctagaaatgtctatgatgtgtgtccactagaagttgattcacaaacgactgctagaatcgcgtgatagggcatcttgaagtttacattgttgtatcgcaaggtactccgatcttaatggatgcgaagtggtacggatgcaatcaagcgcgtgagagcggtacattagagcgttcacctacgctacgctaacgggcgattctgataagaatgcacattgcgtcgattcataagatgtctcgaccgcatgcgcaacttgtgaagtgtctactatccctaagcgcatatctcgcacagtaaccgaatatgtcggcatctgatgttaccgttgagttagtgttcagctcacggaacttattgtatgagtagagatttgtaagagctgttagttagctcgctcagctaatagttgcccacacaacgtcaaattagagaacggtcgtaacattatcggtggttctctaactactatcagtacccacgactcgactctgccgcagctaggtatcgcctgaaagccagtcagcgttaaggagtgctctgaccaggacaacaggcgtagtgagagttacttgttcgttgctcttccgactcggacctgagttcgccaacgacccacttgaggtctgagccggtgaagagaagtaagcatctcgttcgcagcttgccagcactttcagaacatgacccctatttgtttatttttctaaatacattcaaatatgtatccgctcatgagacaataaccctgataaatgcttcaataatattgaaaaaggaagagtggccgcctcggcctaggcttttgcaaagatcgatcaagagacaggatgaggatcgtttcgcatgattgaacaagatggattgcacgcaggttctccggccgcttgggtggagaggctattcggctatgactgggcacaacagacaatcggctgctctgatgccgccgtgttccggctgtcagcgcaggggcgcccggttctttttgtcaagaccgacctgtccggtgccctgaatgaactgcaagacgaggcagcgcggctatcgtggctggccacgacgggcgttccttgcgcagctgtgctcgacgttgtcactgaagcgggaagggactggctgctattgggcgaagtgccggggcaggatctcctgtcatctcaccttgctcctgccgagaaagtatccatcatggctgatgcaatgcggcggctgcatacgcttgatccggctacctgcccattcgaccaccaagcgaaacatcgcatcgagcgagcacgtactcggatggaagccggtcttgtcgatcaggatgatctggacgaagagcatcaggggctcgcgccagccgaactgttcgccaggctcaaggcgagcatgcccgacggcgaggatctcgtcgtgacccatggcgatgcctgcttgccgaatatcatggtggaaaatggccgcttttctggattcatcgactgtggccggctgggtgtggcggaccgctatcaggacatagcgttggctacccgtgatattgctgaagagcttggcggcgaatgggctgaccgcttcctcgtgctttacggtatcgccgctcccgattcgcagcgcatcgccttctatcgccttcttgacgagttcttctgaggtaccatgatgcgtgcatggtagaatgactcttgataacggacttcgactaggcaatatcccttgtcaacttgtcgaggagaaaagtattgactgaagcgctcccggcacaacggccaaagaagtctcagcaatgttcttatttccgaatgacatgcgtctccttgcgggtaaatcgccgaccgcaaaacttaggagccaggatacagataggtctaacttaggttaagggagtaaatcctgggatcgttcagttgtaaccatatacttacgctggggcttctccggcggatgttactgtcaccaaccacgagatttgaagtaaacgcatgattgagcacatagccgcgctatccgacaatctccaaattgataacataccgttccatgaaggccagaattacttaccggccctttccatgcgtgcgccataccgcactctgcgcttatccgtccgaggggagagtgtgcgatcctccgttaagatattctcacgtatgacgtagctatgtattgtgcagaggtagcgaaggcgttgaacacttcacagatggtggggattcgggcaaagggcgtgataacttggggactaacataggcgtaaactacgatggcaccaactcaatcgcagctcgtgcgccctgaatcaacgtactcatctcaactgattctcggcaatctacggagcgacttgattatcaacacctgtctagcagttctaatcttctgccaacatcgtacatagcctccaagagattatcatacctatcggcacagaagtgacacgacgccgaagggtagcggacttctggtcaaccacaattccccaggggacaggtcctgcggtgcgcatcactttgtaagtgcaagcaacccaagtgagcccagcctggactgagctggttcctgtgtcaggtcgaggctggggatgacagctcttgtaaacatagtgatcaagcgtggcgtcgaacggtcgagaaactcatagtacctcgggtagcaacttactcaggttattgcttgaagctgtactatttcaggagcgctgaaggtctcttcttctgtagactgaactcgcaagggtcgtgaagtcggttccttcaatgcttaacaagaacaaaggcttactgtgcagactggaacgcccatctagcggctcgcgtcttgaatgctcggtcccctttgtcattgcggatacaatccatttccctcattcaccagcttgcgaagtctacattgagtagacgaatgcgacctagaagaggtgcgcttcagaacttgtgaggagtggttgatgctctatactccatttggtgtttcgtgcatcaccgcgataggctgacaagaggtcttgaacattgaatagcaaggcacttccggtctcatagaagagagcacgggataaggtacgcgcgtggtacgggaggatcaaggggctacacgatagaaaggcttctccctcactcgctaggaggcaaatgcagaacgctggttactactacgatacgtgaaacttgtccaacggttgcccaaagtgttaagtgtctatcaccctagtgccgtttcccggagaaaacgccaggttgaatccgcatttgaagctacgatggtgaagtctgggtcgagcgcgccgcatgttgattgcgtgagtaggctcgaccaagaaccgctagtagcgtcgctgtagaaatagttctcgacagaccgtcgagtttagaaaatggtagcagcattgttcgcatctcaatcaagtatggattacggtgtttacactgtcctgcggctacccatcgcctgaaatccagctcgtgtcaagccattgcctctccgggacgccgcatgaagtaactacatataccttgcacgggttgactgcggtccgttcagactcgaccaaggacacaatccagcgatcggtgcgggcctcttcgctattacgccag